European Patent Application EP 4 438 729 A2, published October 2, 2024. Title: CRISPR ABASIC RESTRICTED NUCLEOTIDES AND CRISPR ACCURACY VIA ANALOGS. Applicant: CARIBOU BIOSCIENCES, INC. The sequence listing filed with the application follows.

SEQUENCE LISTING (96 sequences)

SEQ ID NO: 1 - RNA, 66 nt, synthetic construct
  misc_feature 1..66: note = Synthetic: tracrRNA
  source 1..66: mol_type = other RNA
agcatagcaagttaaaataaggctagtccgttatcaacttgaaaaagtggcaccgagtcggtgctt

SEQ ID NO: 2 - DNA, 66 bp, synthetic construct
  misc_feature 1..66: note = Synthetic: ch-acr
  misc_feature 1..3: note = DNA
  misc_feature 4..50: note = RNA
  misc_feature 55..59: note = RNA
  misc_feature 60..63: note = DNA
  misc_feature 64..66: note = RNA
  source 1..66: mol_type = other DNA
agcaatccaagttaaaataaggctagtccgttatcaacttgaaaaagtggcaccgagtcggtgctt

SEQ ID NO: 3 - protein, 1368 aa, Streptococcus pyogenes [sequence omitted]

SEQ ID NO: 4 - protein, 11 aa, synthetic construct
  REGION 1..11: note = Synthetic: Nuclear localization sequence (NLS)
GSGSPKKKRKV

SEQ ID NO: 5 - RNA, 36 nt, synthetic construct
  misc_feature 1..36: note = Synthetic: PDCD1 crRNA
  source 1..36: mol_type = other RNA
gtctgggcggtgctacaactgttttagaggattgct

SEQ ID NO: 6 - DNA, 36 bp, synthetic construct
  misc_feature 1..36: note = Synthetic: PDCD1 chRDNA
  misc_feature 1..10: note = DNA
  misc_feature 11..36: note = RNA
  source 1..36: mol_type = other DNA
gtctgggcggtgctacaactgttttagaggattgct

SEQ ID NO: 7 - RNA, 36 nt, synthetic construct
  misc_feature 1..36: note = Synthetic: PDCD1 CABERNT
  modified_base 4: mod_base = OTHER; note = n is abasic ribose site
  source 1..36: mol_type = other RNA
gtcngggcggtgctacaactgttttagaggattgct

SEQ ID NO: 8 - RNA, 36 nt, synthetic construct
  misc_feature 1..36: note = Synthetic: PDCD1 CABERNT
  modified_base 5: mod_base = OTHER; note = n is abasic deoxyribose
  source 1..36: mol_type = other RNA
gtctnggcggtgctacaactgttttagaggattgct

SEQ ID NO: 9 - RNA, 36 nt, synthetic construct
  misc_feature 1..36: note = Synthetic: PDCD1 CABERNT
  modified_base 6: mod_base = OTHER; note = n is abasic deoxyribose
  source 1..36: mol_type = other RNA
gtctgngcggtgctacaactgttttagaggattgct

SEQ ID NO: 10 - RNA, 36 nt, synthetic construct; identical to SEQ ID NO: 7
  misc_feature 1..36: note = Synthetic: PDCD1 CABERNT
  variation 4: note = n is a, c, g, or u
  source 1..36: mol_type = other RNA

SEQ ID NO: 11 - RNA, 36 nt, synthetic construct; identical to SEQ ID NO: 8
  misc_feature 1..36: note = Synthetic: PDCD1 CABERNT
  variation 5: note = n is a, c, g, or u
  source 1..36: mol_type = other RNA

SEQ ID NO: 12 - RNA, 36 nt, synthetic construct; identical to SEQ ID NO: 9
  misc_feature 1..36: note = Synthetic: PDCD1 CABERNT
  variation 6: note = n is a, c, g, or u
  source 1..36: mol_type = other RNA

SEQ ID NO: 13 - RNA, 36 nt, synthetic construct
  misc_feature 1..36: note = Synthetic: TRAC crRNA
  source 1..36: mol_type = other RNA
ttcggaacccaatcactgacgttttagaggattgct

SEQ ID NO: 14 - RNA, 36 nt, synthetic construct
  misc_feature 1..36: note = Synthetic: TRAC CABRNT
  modified_base 20: mod_base = OTHER; note = n is abasic deoxyribose
  source 1..36: mol_type = other RNA
ttcggaacccaatcactgangttttagaggattgct

SEQ ID NO: 15 - RNA, 36 nt, synthetic construct
  misc_feature 1..36: note = Synthetic: TRAC CABRNT
  modified_base 19: mod_base = OTHER; note = n is abasic deoxyribose
  source 1..36: mol_type = other RNA
ttcggaacccaatcactgncgttttagaggattgct

SEQ ID NO: 16 - RNA, 36 nt, synthetic construct
  misc_feature 1..36: note = Synthetic: TRAC CABRNT
  modified_base 18: mod_base = OTHER; note = n is abasic deoxyribose
  source 1..36: mol_type = other RNA
ttcggaacccaatcactnacgttttagaggattgct

SEQ ID NO: 17 - RNA, 36 nt, synthetic construct
  misc_feature 1..36: note = Synthetic: TRAC CABRNT
  modified_base 17: mod_base = OTHER; note = n is abasic deoxyribose
  source 1..36: mol_type = other RNA
ttcggaacccaatcacngacgttttagaggattgct

SEQ ID NO: 18 - RNA, 36 nt, synthetic construct
  misc_feature 1..36: note = Synthetic: TRAC CABRNT
  modified_base 16: mod_base = OTHER; note = n is abasic deoxyribose
  source 1..36: mol_type = other RNA
ttcggaacccaatcantgacgttttagaggattgct

SEQ ID NO: 19 - RNA, 36 nt, synthetic construct
  misc_feature 1..36: note = Synthetic: TRAC CABRNT
  modified_base 15: mod_base = OTHER; note = n is abasic deoxyribose
  source 1..36: mol_type = other RNA
ttcggaacccaatcnctgacgttttagaggattgct

SEQ ID NO: 20 - RNA, 36 nt, synthetic construct
  misc_feature 1..36: note = Synthetic: TRAC CABRNT
  modified_base 14: mod_base = OTHER; note = n is abasic deoxyribose
  source 1..36: mol_type = other RNA
ttcggaacccaatnactgacgttttagaggattgct

SEQ ID NO: 21 - RNA, 36 nt, synthetic construct
  misc_feature 1..36: note = Synthetic: TRAC CABRNT
  modified_base 13: mod_base = OTHER; note = n is abasic deoxyribose
  source 1..36: mol_type = other RNA
ttcggaacccaancactgacgttttagaggattgct

SEQ ID NO: 22 - RNA, 36 nt, synthetic construct
  misc_feature 1..36: note = Synthetic: TRAC CABRNT
  modified_base 12: mod_base = OTHER; note = n is abasic deoxyribose
  source 1..36: mol_type = other RNA
ttcggaacccantcactgacgttttagaggattgct

SEQ ID NO: 23 - RNA, 36 nt, synthetic construct
  misc_feature 1..36: note = Synthetic: TRAC CABRNT
  modified_base 11: mod_base = OTHER; note = n is abasic deoxyribose
  source 1..36: mol_type = other RNA
ttcggaacccnatcactgacgttttagaggattgct

SEQ ID NO: 24 - RNA, 36 nt, synthetic construct
  misc_feature 1..36: note = Synthetic: TRAC CABRNT
  modified_base 10: mod_base = OTHER; note = n is abasic deoxyribose
  source 1..36: mol_type = other RNA
ttcggaaccnaatcactgacgttttagaggattgct

SEQ ID NO: 25 - RNA, 36 nt, synthetic construct
  misc_feature 1..36: note = Synthetic: TRAC CABRNT
  modified_base 9: mod_base = OTHER; note = n is abasic deoxyribose
  source 1..36: mol_type = other RNA
ttcggaacncaatcactgacgttttagaggattgct

SEQ ID NO: 26 - RNA, 36 nt, synthetic construct
  misc_feature 1..36: note = Synthetic: TRAC CABRNT
  modified_base 8: mod_base = OTHER; note = n is abasic deoxyribose
  source 1..36: mol_type = other RNA
ttcggaanccaatcactgacgttttagaggattgct

SEQ ID NO: 27 - RNA, 36 nt, synthetic construct
  misc_feature 1..36: note = Synthetic: TRAC CABRNT
  modified_base 7: mod_base = OTHER; note = n is abasic deoxyribose
  source 1..36: mol_type = other RNA
ttcggancccaatcactgacgttttagaggattgct

SEQ ID NO: 28 - RNA, 36 nt, synthetic construct
  misc_feature 1..36: note = Synthetic: TRAC CABRNT
  modified_base 6: mod_base = OTHER; note = n is abasic deoxyribose
  source 1..36: mol_type = other RNA
ttcggnacccaatcactgacgttttagaggattgct

SEQ ID NO: 29 - RNA, 36 nt, synthetic construct
  misc_feature 1..36: note = Synthetic: TRAC CABRNT
  modified_base 5: mod_base = OTHER; note = n is abasic deoxyribose
  source 1..36: mol_type = other RNA
ttcgnaacccaatcactgacgttttagaggattgct

SEQ ID NO: 30 - RNA, 36 nt, synthetic construct
  misc_feature 1..36: note = Synthetic: TRAC CABRNT
  modified_base 4: mod_base = OTHER; note = n is abasic deoxyribose
  source 1..36: mol_type = other RNA
ttcngaacccaatcactgacgttttagaggattgct

SEQ ID NO: 31 - RNA, 36 nt, synthetic construct
  misc_feature 1..36: note = Synthetic: TRAC CABRNT
  modified_base 3: mod_base = OTHER; note = n is abasic deoxyribose
  source 1..36: mol_type = other RNA
ttnggaacccaatcactgacgttttagaggattgct

SEQ ID NO: 32 - RNA, 36 nt, synthetic construct
  misc_feature 1..36: note = Synthetic: TRAC CABRNT
  modified_base 2: mod_base = OTHER; note = n is abasic deoxyribose
  source 1..36: mol_type = other RNA
tncggaacccaatcactgacgttttagaggattgct

SEQ ID NO: 33 - RNA, 37 nt, synthetic construct
  misc_feature 1..37: note = Synthetic: B2M crRNA
  modified_base 2: mod_base = OTHER; note = n is abasic deoxyribose
  source 1..37: mol_type = other RNA
gntcggaacccaatcactgacgttttagaggattgct

SEQ ID NO: 34 - RNA, 36 nt, synthetic construct
  misc_feature 1..36: note = Synthetic: B2M CABRNT
  source 1..36: mol_type = other RNA
ggccacggagcgagacatctgttttagaggattgct

SEQ ID NO: 35 - RNA, 36 nt, synthetic construct
  misc_feature 1..36: note = Synthetic: B2M CABRNT
  modified_base 20: mod_base = OTHER; note = n is abasic deoxyribose
  source 1..36: mol_type = other RNA
ggccacggagcgagacatcngttttagaggattgct

SEQ ID NO: 36 - RNA, 36 nt, synthetic construct
  misc_feature 1..36: note = Synthetic: B2M CABRNT
  modified_base 19: mod_base = OTHER; note = n is abasic deoxyribose
  source 1..36: mol_type = other RNA
ggccacggagcgagacatntgttttagaggattgct

SEQ ID NO: 37 - RNA, 36 nt, synthetic construct
  misc_feature 1..36: note = Synthetic: B2M CABRNT
  modified_base 18: mod_base = OTHER; note = n is abasic deoxyribose
  source 1..36: mol_type = other RNA
ggccacggagcgagacanctgttttagaggattgct

SEQ ID NO: 38 - RNA, 36 nt, synthetic construct
  misc_feature 1..36: note = Synthetic: B2M CABRNT
  modified_base 17: mod_base = OTHER; note = n is abasic deoxyribose
  source 1..36: mol_type = other RNA
ggccacggagcgagacntctgttttagaggattgct

SEQ ID NO: 39 - RNA, 36 nt, synthetic construct
  misc_feature 1..36: note = Synthetic: B2M CABRNT
  modified_base 16: mod_base = OTHER; note = n is abasic deoxyribose
  source 1..36: mol_type = other RNA
ggccacggagcgaganatctgttttagaggattgct

SEQ ID NO: 40 - RNA, 36 nt, synthetic construct
  misc_feature 1..36: note = Synthetic: B2M CABRNT
  modified_base 15: mod_base = OTHER; note = n is abasic deoxyribose
  source 1..36: mol_type = other RNA
ggccacggagcgagncatctgttttagaggattgct

SEQ ID NO: 41 - RNA, 36 nt, synthetic construct
  misc_feature 1..36: note = Synthetic: B2M CABRNT
  modified_base 14: mod_base = OTHER; note = n is abasic deoxyribose
  source 1..36: mol_type = other RNA
ggccacggagcganacatctgttttagaggattgct

SEQ ID NO: 42 - RNA, 36 nt, synthetic construct
  misc_feature 1..36: note = Synthetic: B2M CABRNT
  modified_base 13: mod_base = OTHER; note = n is abasic deoxyribose
  source 1..36: mol_type = other RNA
ggccacggagcgngacatctgttttagaggattgct

SEQ ID NO: 43 - RNA, 36 nt, synthetic construct
  misc_feature 1..36: note = Synthetic: B2M CABRNT
  modified_base 12: mod_base = OTHER; note = n is abasic deoxyribose
  source 1..36: mol_type = other RNA
ggccacggagcnagacatctgttttagaggattgct

SEQ ID NO: 44 - RNA, 36 nt, synthetic construct
  misc_feature 1..36: note = Synthetic: B2M CABRNT
  modified_base 11: mod_base = OTHER; note = n is abasic deoxyribose
  source 1..36: mol_type = other RNA
ggccacggagngagacatctgttttagaggattgct

SEQ ID NO: 45 - RNA, 36 nt, synthetic construct
  misc_feature 1..36: note = Synthetic: B2M CABRNT
  modified_base 10: mod_base = OTHER; note = n is abasic deoxyribose
  source 1..36: mol_type = other RNA
ggccacggancgagacatctgttttagaggattgct

SEQ ID NO: 46 - RNA, 36 nt, synthetic construct
  misc_feature 1..36: note = Synthetic: B2M CABRNT
  modified_base 9: mod_base = OTHER; note = n is abasic deoxyribose
  source 1..36: mol_type = other RNA
ggccacggngcgagacatctgttttagaggattgct

SEQ ID NO: 47 - RNA, 36 nt, synthetic construct
  misc_feature 1..36: note = Synthetic: B2M CABRNT
  modified_base 8: mod_base = OTHER; note = n is abasic deoxyribose
  source 1..36: mol_type = other RNA
ggccacgnagcgagacatctgttttagaggattgct

SEQ ID NO: 48 - RNA, 36 nt, synthetic construct
  misc_feature 1..36: note = Synthetic: B2M CABRNT
  modified_base 7: mod_base = OTHER; note = n is abasic deoxyribose
  source 1..36: mol_type = other RNA
ggccacngagcgagacatctgttttagaggattgct

SEQ ID NO: 49 - RNA, 36 nt, synthetic construct
  misc_feature 1..36: note = Synthetic: B2M CABRNT
  modified_base 6: mod_base = OTHER; note = n is abasic deoxyribose
  source 1..36: mol_type = other RNA
ggccanggagcgagacatctgttttagaggattgct

SEQ ID NO: 50 - RNA, 36 nt, synthetic construct
  misc_feature 1..36: note = Synthetic: B2M CABRNT
  modified_base 5: mod_base = OTHER; note = n is abasic deoxyribose
  source 1..36: mol_type = other RNA
ggccncggagcgagacatctgttttagaggattgct

SEQ ID NO: 51 - RNA, 36 nt, synthetic construct
  misc_feature 1..36: note = Synthetic: B2M CABRNT
  modified_base 4: mod_base = OTHER; note = n is abasic deoxyribose
  source 1..36: mol_type = other RNA
ggcnacggagcgagacatctgttttagaggattgct

SEQ ID NO: 52 - RNA, 36 nt, synthetic construct
  misc_feature 1..36: note = Synthetic: B2M CABRNT
  modified_base 3: mod_base = OTHER; note = n is abasic deoxyribose
  source 1..36: mol_type = other RNA
ggncacggagcgagacatctgttttagaggattgct

SEQ ID NO: 53 - RNA, 36 nt, synthetic construct
  misc_feature 1..36: note = Synthetic: B2M CABRNT
  modified_base 2: mod_base = OTHER; note = n is abasic deoxyribose
  source 1..36: mol_type = other RNA
gnccacggagcgagacatctgttttagaggattgct

SEQ ID NO: 54 - RNA, 37 nt, synthetic construct
  misc_feature 1..37: note = Synthetic: B2M CABRNT
  modified_base 2: mod_base = OTHER; note = n is abasic deoxyribose
  source 1..37: mol_type = other RNA
gngccacggagcgagacatctgttttagaggattgct

SEQ ID NO: 55 - RNA, 36 nt, synthetic construct
  misc_feature 1..36: note = Synthetic: AAVS1 crRNA
  source 1..36: mol_type = other RNA
ggggccactagggacaggatgttttagaggattgct

SEQ ID NO: 56 - DNA, 36 bp, synthetic construct
  misc_feature 1..36: note = Synthetic: AAVS1 CABRNT
  misc_feature 1..2: note = DNA
  modified_base 3: mod_base = OTHER; note = n is abasic deoxyribose
  misc_feature 4..10: note = DNA
  misc_feature 11..36: note = RNA
  source 1..36: mol_type = other DNA
ggngccactagggacaggatgttttagaggattgct

SEQ ID NO: 57 - DNA, 36 bp, synthetic construct; identical to SEQ ID NO: 56
  misc_feature 1..36: note = Synthetic: AAVS1 CABRNT
  misc_feature 1..2: note = DNA
  modified_base 3: mod_base = OTHER; note = n is abasic deoxyribose
  misc_feature 4..5: note = DNA
  misc_feature 6..36: note = RNA
  source 1..36: mol_type = other DNA

SEQ ID NO: 58 - DNA, 36 bp, synthetic construct; identical to SEQ ID NO: 56
  misc_feature 1..36: note = Synthetic: AAVS1 CABRNT
  misc_feature 1..2: note = RNA
  modified_base 3: mod_base = OTHER; note = n is abasic deoxyribose
  misc_feature 4..10: note = DNA
  misc_feature 11..36: note = RNA
  source 1..36: mol_type = other DNA

SEQ ID NO: 59 - DNA, 36 bp, synthetic construct; identical to SEQ ID NO: 56
  misc_feature 1..36: note = Synthetic: AAVS1 CABRNT
  misc_feature 1..2: note = DNA
  modified_base 3: mod_base = OTHER; note = n is abasic deoxyribose
  misc_feature 4: note = RNA
  misc_feature 5..12: note = DNA
  misc_feature 13..36: note = RNA
  source 1..36: mol_type = other DNA

SEQ ID NO: 60 - DNA, 36 bp, synthetic construct; identical to SEQ ID NO: 56
  misc_feature 1..36: note = Synthetic: AAVS1 CABRNT
  misc_feature 1: note = RNA
  misc_feature 2: note = DNA
  modified_base 3: mod_base = OTHER; note = n is abasic deoxyribose
  misc_feature 4: note = RNA
  misc_feature 5..9: note = DNA
  misc_feature 10..13: note = RNA
  misc_feature 14: note = DNA
  misc_feature 15..16: note = RNA
  misc_feature 17..18: note = DNA
  misc_feature 19..36: note = DNA
  source 1..36: mol_type = other DNA

SEQ ID NO: 61 - DNA, 23 bp, Homo sapiens
  misc_feature 1..23: note = PDCD1 target
  source 1..23: mol_type = genomic DNA
gtctgggcggtgctacaactggg

SEQ ID NO: 62 - DNA, 23 bp, Homo sapiens
  misc_feature 1..23: note = PDCD1 off-target
  source 1..23: mol_type = genomic DNA
aacggggcggtactacaacttgg

SEQ ID NO: 63 - DNA, 23 bp, Homo sapiens
  misc_feature 1..23: note = PDCD1 off-target
  source 1..23: mol_type = genomic DNA
tgtctggtggtgctacaacttgg

SEQ ID NO: 64 - DNA, 23 bp, Homo sapiens
  misc_feature 1..23: note = PDCD1 off-target
  source 1..23: mol_type = genomic DNA
acctggacggtgatacaacccgg

SEQ ID NO: 65 - RNA, 16 nt, synthetic construct
  misc_feature 1..16: note = Synthetic: CRISPR repeat
  source 1..16: mol_type = other RNA
gttttagaggattgct

SEQ ID NO: 66 - DNA, 52 bp, synthetic construct
  misc_feature 1..52: note = Synthetic: Oligo
  source 1..52: mol_type = other DNA
cactctttccctacacgacgctcttccgatctttatgcacagggtggaacaa

SEQ ID NO: 67 - DNA, 48 bp, synthetic construct
  misc_feature 1..48: note = Synthetic: Oligo
  source 1..48: mol_type = other DNA
ggagttcagacgtgtgctcttccgatctgccaggttgagcaggtagat

SEQ ID NO: 68 - DNA, 23 bp, Homo sapiens
  misc_feature 1..23: note = TRAC target
  source 1..23: mol_type = genomic DNA
ttcggaacccaatcactgacagg

SEQ ID NO: 69 - DNA, 23 bp, Homo sapiens
  misc_feature 1..23: note = B2M target
  source 1..23: mol_type = genomic DNA
ggccacggagcgagacatctcgg

SEQ ID NO: 70 - DNA, 23 bp, Homo sapiens
  misc_feature 1..23: note = AAVS1 target
  source 1..23: mol_type = genomic DNA
ggggccactagggacaggattgg

SEQ ID NO: 71 - DNA, 23 bp, Homo sapiens
  misc_feature 1..23: note = AAVS1 off-target
  source 1..23: mol_type = genomic DNA
gggaccatcagggacaggatggg

SEQ ID NO: 72 - DNA, 23 bp, Homo sapiens
  misc_feature 1..23: note = AAVS1 off-target
  source 1..23: mol_type = genomic DNA
ggggcttctaaggacaggatggg

SEQ ID NO: 73 - DNA, 23 bp, Homo sapiens
  misc_feature 1..23: note = AAVS1 off-target
  source 1..23: mol_type = genomic DNA
gaggccaccagggacaggctggg

SEQ ID NO: 74 - DNA, 23 bp, Homo sapiens
  misc_feature 1..23: note = AAVS1 off-target
  source 1..23: mol_type = genomic DNA
ggggccaattaggacaggatggg

SEQ ID NO: 75 - DNA, 23 bp, Homo sapiens
  misc_feature 1..23: note = AAVS1 off-target
  source 1..23: mol_type = genomic DNA
atggccactaaggacaggaaagg

SEQ ID NO: 76 - DNA, 23 bp, Homo sapiens
  misc_feature 1..23: note = B2M off-target
  source 1..23: mol_type = genomic DNA
ggcgacagaacgagacatctcgg

SEQ ID NO: 77 - RNA, 36 nt, synthetic construct; identical to SEQ ID NO: 5
  misc_feature 1..36: note = Synthetic: PDCD1 CAVA
  source 1..36: mol_type = other RNA

SEQ ID NO: 78 - RNA, 36 nt, synthetic construct; identical to SEQ ID NO: 5
  misc_feature 1..36: note = Synthetic: PDCD1 CAVA
  source 1..36: mol_type = other RNA

SEQ ID NO: 79 - RNA, 36 nt, synthetic construct; identical to SEQ ID NO: 5
  misc_feature 1..36: note = Synthetic: PDCD1 CAVA
  source 1..36: mol_type = other RNA

SEQ ID NO: 80 - RNA, 36 nt, synthetic construct; identical to SEQ ID NO: 5
  misc_feature 1..36: note = Synthetic: PDCD1 CAVA
  source 1..36: mol_type = other RNA

SEQ ID NO: 81 - RNA, 36 nt, synthetic construct; identical to SEQ ID NO: 5
  misc_feature 1..36: note = Synthetic: PDCD1 CAVA
  source 1..36: mol_type = other RNA

SEQ ID NO: 82 - RNA, 36 nt, synthetic construct; identical to SEQ ID NO: 5
  misc_feature 1..36: note = Synthetic: PDCD1 CAVA
  source 1..36: mol_type = other RNA

SEQ ID NO: 83 - RNA, 36 nt, synthetic construct; identical to SEQ ID NO: 5
  misc_feature 1..36: note = Synthetic: PDCD1 CAVA
  source 1..36: mol_type = other RNA

SEQ ID NO: 84 - RNA, 36 nt, synthetic construct
  misc_feature 1..36: note = Synthetic: PDCD1 CAVA
  modified_base 3..4: mod_base = OTHER; note = n is inosine
  source 1..36: mol_type = other RNA
gtnngggcggtgctacaactgttttagaggattgct

SEQ ID NO: 85 - RNA, 36 nt, synthetic construct
  misc_feature 1..36: note = Synthetic: PDCD1 CAVA
  modified_base 5..6: mod_base = OTHER; note = n is inosine
  source 1..36: mol_type = other RNA
gtctnngcggtgctacaactgttttagaggattgct

SEQ ID NO: 86 - RNA, 36 nt, synthetic construct
  misc_feature 1..36: note = Synthetic: PDCD1 CAVA
  modified_base 2..3: mod_base = OTHER; note = n is deoxyinosine
  source 1..36: mol_type = other RNA
gnntgggcggtgctacaactgttttagaggattgct

SEQ ID NO: 87 - RNA, 36 nt, synthetic construct
  misc_feature 1..36: note = Synthetic: PDCD1 CAVA
  modified_base 4..5: mod_base = OTHER; note = n is deoxyinosine
  source 1..36: mol_type = other RNA
gtcnnggcggtgctacaactgttttagaggattgct

SEQ ID NO: 88 - RNA, 36 nt, synthetic construct
  misc_feature 1..36: note = Synthetic: PDCD1 CAVA
  modified_base 6..7: mod_base = OTHER; note = n is deoxyinosine
  source 1..36: mol_type = other RNA
gtctgnncggtgctacaactgttttagaggattgct

SEQ ID NO: 89 - RNA, 36 nt, synthetic construct
  misc_feature 1..36: note = Synthetic: PDCD1 CAVA
  modified_base 8..9: mod_base = OTHER; note = n is deoxyinosine
  source 1..36: mol_type = other RNA
gtctgggnngtgctacaactgttttagaggattgct

SEQ ID NO: 90 - RNA, 36 nt, synthetic construct
  misc_feature 1..36: note = Synthetic: PDCD1 CAVA
  modified_base 10..11: mod_base = OTHER; note = n is deoxyinosine
  source 1..36: mol_type = other RNA
gtctgggcgnngctacaactgttttagaggattgct

SEQ ID NO: 91 - RNA, 36 nt, synthetic construct
  misc_feature 1..36: note = Synthetic: Cas9 cr-element
  variation 1..20: note = n is a, c, g, or u
  source 1..36: mol_type = other RNA
nnnnnnnnnnnnnnnnnnnngttttagaggattgct

SEQ ID NO: 92 - RNA, 40 nt, synthetic construct
  misc_feature 1..40: note = Synthetic: Cas12a cr-element
  variation 21..40: note = n is a, c, g, or u
  source 1..40: mol_type = other RNA
taatttctactcttgtagatnnnnnnnnnnnnnnnnnnnn

SEQ ID NO: 93 - protein, 117 aa, synthetic construct
  REGION 1..117: note = Synthetic: anti-BCMA heavy chain variable region
QVQLVQSGAEVKKPGSSVKVSCKASGYTFTSYVMHWVRQAPGQGLEWMGYIIPYNDATKYNEKFKGRVTITADKSTSTAYMELSSLRSEDTAVYYCARYNYDGYFDVWGQGTLVTVS

SEQ ID NO: 94 - protein, 107 aa, synthetic construct
  REGION 1..107: note = Synthetic: anti-BCMA light chain variable region
EIVLTQSPATLSLSPGERATLSCRASQSISDYLHWYQQKPGQAPRLLIYYASQSITGIPARFSGSGSGTDFTLTISSLEPEDFAVYYCQNGHSFPPTFGGGTKVEIK

SEQ ID NO: 95 - protein, 15 aa, synthetic construct
  REGION 1..15: note = Synthetic: BCMA scFv linker
GGGGSGGGGSGGGGS

SEQ ID NO: 96 - protein, 240 aa, synthetic construct
  REGION 1..240: note = Synthetic: BCMA scFv
QVQLVQSGAEVKKPGSSVKVSCKASGYTFTSYVMHWVRQAPGQGLEWMGYIIPYNDATKYNEKFKGRVTITADKSTSTAYMELSSLRSEDTAVYYCARYNYDGYFDVWGQGTLVTVSSGGGGSGGGGSGGGGSEIVLTQSPATLSLSPGERATLSCRASQSISDYLHWYQQKPGQAPRLLIYYASQSITGIPARFSGSGSGTDFTLTISSLEPEDFAVYYCQNGHSFPPTFGGGTKVEIK